European Patent Specification EP 3 658 566 B1, published July 19, 2023. Title: Side-Chain Modified Ergosterol and Stigmasterol Derivatives as Liver X Receptor modulators. Applicant: Ospedale San Raffaele. The sequence listing filed with the application follows.

SEQUENCE LISTING (14 sequences)

SEQ ID NO: 1 - DNA, 21 bp, Artificial Sequence
  GAPDH primer Forward
acatcatccctgcctctactg

SEQ ID NO: 2 - DNA, 20 bp, Artificial Sequence
  GAPDH primer Reverse
accacctggtgctcagtgta

SEQ ID NO: 3 - DNA, 19 bp, Artificial Sequence
  ABCA1 primer Forward
ccaggccagtacggaattc

SEQ ID NO: 4 - DNA, 19 bp, Artificial Sequence
  ABCA1 primer Reverse
cctcgccaaaccagtagga

SEQ ID NO: 5 - DNA, 14 bp, Artificial Sequence
  SREBP-1c prmier Forward
ggcgggcgcagatc

SEQ ID NO: 6 - DNA, 24 bp, Artificial Sequence
  SREBP-1c primer Reverse
ttgttgataagctgaagcatgtct

SEQ ID NO: 7 - DNA, 25 bp, Artificial Sequence
  MCP-1 primer Forward
agaagctgtgatcttcaagaccatt

SEQ ID NO: 8 - DNA, 20 bp, Artificial Sequence
  MCP-1 primer Reverse
tgcttgtccaggtggtccat

SEQ ID NO: 9 - DNA, 19 bp, Artificial Sequence
  FAS primer Forward
acagcggggaatgggtact

SEQ ID NO: 10 - DNA, 20 bp, Artificial Sequence
  FAS primer Reverse
gactggtacaacgagcggat

SEQ ID NO: 11 - DNA, 30 bp, Artificial Sequence
  SCD1 primer Forward
ttcagaaacacatgctgatcctcataattc

SEQ ID NO: 12 - DNA, 30 bp, Artificial Sequence
  SCD1 primer Reverse
attaagcaccacagcatatcgcaagaaagt

SEQ ID NO: 13 - DNA, 20 bp, Artificial Sequence
  TNF alpha primer Forward
tcttctcgaaccccgagtga

SEQ ID NO: 14 - DNA, 19 bp, Artificial Sequence
  TNF alpha primer Reverse
cctctgatggcaccaccag